European Patent Application EP 4 361 167 A1, published May 1, 2024. Title: INSECT NEUROPEPTIDES 7. Applicant: SOLASTA Bio Limited. The sequence listing filed with the application follows.

SEQUENCE LISTING (16 sequences)

SEQ ID NO: 1 - protein, 7 aa, synthetic construct
  source 1..7: note = Z peptide
PAFSSWG

SEQ ID NO: 2 - protein, 7 aa, synthetic construct
  source 1..7: note = SB-P-66
  MOD_RES 7: note = glycinamide
PAFSSWG

SEQ ID NO: 3 - protein, 11 aa, synthetic construct
  source 1..11: note = SB-P-47
  MOD_RES 11: note = leucinamide
  MOD_RES 1: note = pyroglutamyl-alanine
AIMARPQVPRL

SEQ ID NO: 4 - protein, 8 aa, synthetic construct
  source 1..8: note = SB-P-49
  MOD_RES 8: note = leucinamide
SVPFKPRL

SEQ ID NO: 5 - protein, 19 aa, synthetic construct
  source 1..19: note = SB-P-51
  MOD_RES 19: note = leucinamide
LRQLQSNGEPAYRVRTPRL

SEQ ID NO: 6 - protein, 16 aa, synthetic construct
  source 1..16: note = SB-P-80
  MOD_RES 16: note = leucinamide
NADEDQQQSVDFTPRL

SEQ ID NO: 7 - protein, 10 aa, synthetic construct
  source 1..10: note = SB-P-81
  MOD_RES 10: note = leucinamide
GGSMTFSPRL

SEQ ID NO: 8 - protein, 8 aa, synthetic construct
  source 1..8: note = SB-P-70
  MOD_RES 8: note = glycinamide
KVKFSAWG

SEQ ID NO: 9 - protein, 10 aa, synthetic construct
  source 1..10: note = SB-P-65
  MOD_RES 10: note = glycinamide
RQKTVFSSWG

SEQ ID NO: 10 - protein, 12 aa, synthetic construct
  source 1..12: note = SB-P-46
  MOD_RES 12: note = leucinamide
SPPYSPPFSPRL

SEQ ID NO: 11 - protein, 9 aa, synthetic construct
  source 1..9: note = SB-P-86
  MOD_RES 9: note = glycinamide
  MOD_RES 1: note = pyroglutamyl-leucine
LTFTSSWGG

SEQ ID NO: 12 - protein, 8 aa, synthetic construct
  source 1..8: note = SB-P-039
  MOD_RES 1: note = palmitoyl-glutamine
  MOD_RES 8: note = tryptophanamide
QLTFSPDW

SEQ ID NO: 13 - protein, 7 aa, synthetic construct
  source 1..7: note = SB-P-042
  MOD_RES 1: note = pyroglutamyl-leucine
  MOD_RES 7: note = tryptophanamide
LTFSPDW

SEQ ID NO: 14 - protein, 6 aa, synthetic construct
  source 1..6: note = SB-P-69
  MOD_RES 6: note = glycinamide
NFSPWG

SEQ ID NO: 15 - protein, 19 aa, synthetic construct
  source 1..19: note = SB-P-48
  MOD_RES 19: note = leucinamide
EQNVQSNGEPAYRVRTPRL

SEQ ID NO: 16 - protein, 8 aa, synthetic construct
  source 1..8: note = SB-P-41
  MOD_RES 8: note = tryptophanamide
QLTFSPDW